European Patent Application EP 4 534 680 A1, published April 9, 2025. Title: Polynucleotide. Applicant: 国立大学法人東海国立大学機構. The sequence listing filed with the application follows.

SEQUENCE LISTING (35 sequences)

SEQ ID NO: 1 - protein, 267 aa, synthetic construct
  REGION 1..267: note = CD19scFv
MLLLVTSLLLCELPHPAFLLIPDIQMTQTTSSLSASLGDRVTISCRASQDISKYLNWYQQKPDGTVKLLIYHTSRLHSGVPSRFSGSGSGTDYSLTISNLEQEDIATYFCQQGNTLPYTFGGGTKLEITGSTSGSGKPGSGEGSTKGEVKLQESGPGLVAPSQSLSVTCTVSGVSLPDYGVSWIRQPPRKGLEWLGVIWGSETTYYNSALKSRLTIIKDNSKSQVFLKMNSLQTDDTAIYYCAKHYYYGGSYAMDYWGQGTSVTVSS

SEQ ID NO: 2 - protein, 12 aa, synthetic construct
  REGION 1..12: note = IgG4 hinge
ESKYGPPCPPCP

SEQ ID NO: 3 - protein, 28 aa, synthetic construct
  REGION 1..28: note = CD28 transmenbrane domain
MFWVLVVVGGVLACYSLLVTVAFIIFWV

SEQ ID NO: 4 - protein, 41 aa, synthetic construct
  REGION 1..41: note = CD28 intracellular domain
RSKRSRLLHSDYMNMTPRRPGPTRKHYQPYAPPRDFAAYRS

SEQ ID NO: 5 - protein, 112 aa, synthetic construct
  REGION 1..112: note = CD3z intracellular domain
RVKFSRSADAPAYQQGQNQLYNELNLGRREEYDVLDKRRGRDPEMGGKPRRKNPQEGLYNELQKDKMAEAYSEIGMKGERRRGKGHDGLYQGLSTATKDTYDALHMQALPPR

SEQ ID NO: 6 - protein, 19 aa, synthetic construct
  REGION 1..19: note = T2A
EGRGSLLTCGDVEENPGPR

SEQ ID NO: 7 - protein, 357 aa, synthetic construct
  REGION 1..357: note = truncated EGFR
MLLLVTSLLLCELPHPAFLLIPRKVCNGIGIGEFKDSLSINATNIKHFKNCTSISGDLHILPVAFRGDSFTHTPPLDPQELDILKTVKEITGFLLIQAWPENRTDLHAFENLEIIRGRTKQHGQFSLAVVSLNITSLGLRSLKEISDGDVIISGNKNLCYANTINWKKLFGTSGQKTKIISNRGENSCKATGQVCHALCSPEGCWGPEPRDCVSCRNVSRGRECVDKCNLLEGEPREFVENSECIQCHPECLPQAMNITCTGRGPDNCIQCAHYIDGPHCVKTCPAGVMGENNTLVWKYADAGHVCHLCHPNCTYGCTGPGLEGCPTNGPKIPSIATGMVGALLLLLVVALGIGLFM

SEQ ID NO: 8 - protein, 841 aa, synthetic construct
  REGION 1..841: note = CAR
MLLLVTSLLLCELPHPAFLLIPDIQMTQTTSSLSASLGDRVTISCRASQDISKYLNWYQQKPDGTVKLLIYHTSRLHSGVPSRFSGSGSGTDYSLTISNLEQEDIATYFCQQGNTLPYTFGGGTKLEITGSTSGSGKPGSGEGSTKGEVKLQESGPGLVAPSQSLSVTCTVSGVSLPDYGVSWIRQPPRKGLEWLGVIWGSETTYYNSALKSRLTIIKDNSKSQVFLKMNSLQTDDTAIYYCAKHYYYGGSYAMDYWGQGTSVTVSSESKYGPPCPPCPMFWVLVVVGGVLACYSLLVTVAFIIFWVRSKRSRLLHSDYMNMTPRRPGPTRKHYQPYAPPRDFAAYRSRVKFSRSADAPAYQQGQNQLYNELNLGRREEYDVLDKRRGRDPEMGGKPRRKNPQEGLYNELQKDKMAEAYSEIGMKGERRRGKGHDGLYQGLSTATKDTYDALHMQALPPRLEGGGEGRGSLLTCGDVEENPGPRMLLLVTSLLLCELPHPAFLLIPRKVCNGIGIGEFKDSLSINATNIKHFKNCTSISGDLHILPVAFRGDSFTHTPPLDPQELDILKTVKEITGFLLIQAWPENRTDLHAFENLEIIRGRTKQHGQFSLAVVSLNITSLGLRSLKEISDGDVIISGNKNLCYANTINWKKLFGTSGQKTKIISNRGENSCKATGQVCHALCSPEGCWGPEPRDCVSCRNVSRGRECVDKCNLLEGEPREFVENSECIQCHPECLPQAMNITCTGRGPDNCIQCAHYIDGPHCVKTCPAGVMGENNTLVWKYADAGHVCHLCHPNCTYGCTGPGLEGCPTNGPKIPSIATGMVGALLLLLVVALGIGLFM

SEQ ID NO: 9 - DNA, 801 bp, synthetic construct
  misc_feature 1..801: note = CD19scFv
  source 1..801: mol_type = other DNA
atgctgctgctggtgaccagcctgctgctgtgcgagctgccccaccccgcctttctgctgatccccgacatccagatgacccagaccacctccagcctgagcgccagcctgggcgaccgggtgaccatcagctgccgggccagccaggacatcagcaagtacctgaactggtatcagcagaagcccgacggcaccgtcaagctgctgatctaccacaccagccggctgcacagcggcgtgcccagccggtttagcggcagcggctccggcaccgactacagcctgaccatctccaacctggaacaggaagatatcgccacctacttttgccagcagggcaacacactgccctacacctttggcggcggaacaaagctggaaatcaccggcagcacctccggcagcggcaagcctggcagcggcgagggcagcaccaagggcgaggtgaagctgcaggaaagcggccctggcctggtggcccccagccagagcctgagcgtgacctgcaccgtgagcggcgtgagcctgcccgactacggcgtgagctggatccggcagccccccaggaagggcctggaatggctgggcgtgatctggggcagcgagaccacctactacaacagcgccctgaagagccggctgaccatcatcaaggacaacagcaagagccaggtgttcctgaagatgaacagcctgcagaccgacgacaccgccatctactactgcgccaagcactactactacggcggcagctacgccatggactactggggccagggcaccagcgtgaccgtgagcagc

SEQ ID NO: 10 - DNA, 36 bp, synthetic construct
  misc_feature 1..36: note = IgG4 hinge
  source 1..36: mol_type = other DNA
gaatctaagtacggaccgccctgccccccttgccct

SEQ ID NO: 11 - DNA, 84 bp, synthetic construct
  misc_feature 1..84: note = CD28 transmembrane domain
  source 1..84: mol_type = other DNA
atgttctgggtgctggtggtggtcggaggcgtgctggcctgctacagcctgctggtcaccgtggccttcatcatcttttgggtg

SEQ ID NO: 12 - DNA, 123 bp, synthetic construct
  misc_feature 1..123: note = CD28 intracellular domain
  source 1..123: mol_type = other DNA
cggagcaagcggagcagaggcggccacagcgactacatgaacatgacccccagacggcctggccccacccggaagcactaccagccctacgccccacccagggactttgccgcctaccggtcc

SEQ ID NO: 13 - DNA, 336 bp, synthetic construct
  misc_feature 1..336: note = CD3z intracellular domain
  source 1..336: mol_type = other DNA
cgggtgaagttcagcagaagcgccgacgcccctgcctaccagcagggccagaatcagctgtacaacgagctgaacctgggcagaagggaagagtacgacgtcctggataagcggagaggccgggaccctgagatgggcggcaagcctcggcggaagaacccccaggaaggcctgtataacgaactgcagaaagacaagatggccgaggcctacagcgagatcggcatgaagggcgagcggaggcggggcaagggccacgacggcctgtatcagggcctgtccaccgccaccaaggatacctacgacgccctgcacatgcaggccctgcccccaagg

SEQ ID NO: 14 - DNA, 57 bp, synthetic construct
  misc_feature 1..57: note = T2A
  source 1..57: mol_type = other DNA
gagggcagaggaagtcttctaacatgcggtgacgtggaggagaatcccggccctagg

SEQ ID NO: 15 - DNA, 1071 bp, synthetic construct
  misc_feature 1..1071: note = truncated EGFR
  source 1..1071: mol_type = other DNA
atgcttctcctggtgacaagccttctgctctgtgagttaccacacccagcattcctcctgatcccacgcaaagtgtgtaacggaataggtattggtgaatttaaagactcactctccataaatgctacgaatattaaacacttcaaaaactgcacctccatcagtggcgatctccacatcctgccggtggcatttaggggtgactccttcacacatactcctcctctggatccacaggaactggatattctgaaaaccgtaaaggaaatcacagggtttttgctgattcaggcttggcctgaaaacaggacggacctccatgcctttgagaacctagaaatcatacgcggcaggaccaagcaacatggtcagttttctcttgcagtcgtcagcctgaacataacatccttgggattacgctccctcaaggagataagtgatggagatgtgataatttcaggaaacaaaaatttgtgctatgcaaatacaataaactggaaaaaactgtttgggacctccggtcagaaaaccaaaattataagcaacagaggtgaaaacagctgcaaggccacaggccaggtctgccatgccttgtgctcccccgagggctgctggggcccggagcccagggactgcgtctcttgccggaatgtcagccgaggcagggaatgcgtggacaagtgcaaccttctggagggtgagccaagggagtttgtggagaactctgagtgcatacagtgccacccagagtgcctgcctcaggccatgaacatcacctgcacaggacggggaccagacaactgtatccagtgtgcccactacattgacggcccccactgcgtcaagacctgcccggcaggagtcatgggagaaaacaacaccctggtctggaagtacgcagacgccggccatgtgtgccacctgtgccatccaaactgcacctacggatgcactgggccaggtcttgaaggctgtccaacgaatgggcctaagatcccgtccatcgccactgggatggtgggggccctcctcttgctgctggtggtggccctggggatcggcctcttcatg

SEQ ID NO: 16 - DNA, 2526 bp, synthetic construct
  misc_feature 1..2526: note = CAR
  source 1..2526: mol_type = other DNA
atgctgctgctggtgaccagcctgctgctgtgcgagctgccccaccccgcctttctgctgatccccgacatccagatgacccagaccacctccagcctgagcgccagcctgggcgaccgggtgaccatcagctgccgggccagccaggacatcagcaagtacctgaactggtatcagcagaagcccgacggcaccgtcaagctgctgatctaccacaccagccggctgcacagcggcgtgcccagccggtttagcggcagcggctccggcaccgactacagcctgaccatctccaacctggaacaggaagatatcgccacctacttttgccagcagggcaacacactgccctacacctttggcggcggaacaaagctggaaatcaccggcagcacctccggcagcggcaagcctggcagcggcgagggcagcaccaagggcgaggtgaagctgcaggaaagcggccctggcctggtggcccccagccagagcctgagcgtgacctgcaccgtgagcggcgtgagcctgcccgactacggcgtgagctggatccggcagccccccaggaagggcctggaatggctgggcgtgatctggggcagcgagaccacctactacaacagcgccctgaagagccggctgaccatcatcaaggacaacagcaagagccaggtgttcctgaagatgaacagcctgcagaccgacgacaccgccatctactactgcgccaagcactactactacggcggcagctacgccatggactactggggccagggcaccagcgtgaccgtgagcagcgaatctaagtacggaccgccctgccccccttgccctatgttctgggtgctggtggtggtcggaggcgtgctggcctgctacagcctgctggtcaccgtggccttcatcatcttttgggtgcggagcaagcggagcagaggcggccacagcgactacatgaacatgacccccagacggcctggccccacccggaagcactaccagccctacgccccacccagggactttgccgcctaccggtcccgggtgaagttcagcagaagcgccgacgcccctgcctaccagcagggccagaatcagctgtacaacgagctgaacctgggcagaagggaagagtacgacgtcctggataagcggagaggccgggaccctgagatgggcggcaagcctcggcggaagaacccccaggaaggcctgtataacgaactgcagaaagacaagatggccgaggcctacagcgagatcggcatgaagggcgagcggaggcggggcaagggccacgacggcctgtatcagggcctgtccaccgccaccaaggatacctacgacgccctgcacatgcaggccctgcccccaaggctcgagggcggcggagagggcagaggaagtcttctaacatgcggtgacgtggaggagaatcccggccctaggatgcttctcctggtgacaagccttctgctctgtgagttaccacacccagcattcctcctgatcccacgcaaagtgtgtaacggaataggtattggtgaatttaaagactcactctccataaatgctacgaatattaaacacttcaaaaactgcacctccatcagtggcgatctccacatcctgccggtggcatttaggggtgactccttcacacatactcctcctctggatccacaggaactggatattctgaaaaccgtaaaggaaatcacagggtttttgctgattcaggcttggcctgaaaacaggacggacctccatgcctttgagaacctagaaatcatacgcggcaggaccaagcaacatggtcagttttctcttgcagtcgtcagcctgaacataacatccttgggattacgctccctcaaggagataagtgatggagatgtgataatttcaggaaacaaaaatttgtgctatgcaaatacaataaactggaaaaaactgtttgggacctccggtcagaaaaccaaaattataagcaacagaggtgaaaacagctgcaaggccacaggccaggtctgccatgccttgtgctcccccgagggctgctggggcccggagcccagggactgcgtctcttgccggaatgtcagccgaggcagggaatgcgtggacaagtgcaaccttctggagggtgagccaagggagtttgtggagaactctgagtgcatacagtgccacccagagtgcctgcctcaggccatgaacatcacctgcacaggacggggaccagacaactgtatccagtgtgcccactacattgacggcccccactgcgtcaagacctgcccggcaggagtcatgggagaaaacaacaccctggtctggaagtacgcagacgccggccatgtgtgccacctgtgccatccaaactgcacctacggatgcactgggccaggtcttgaaggctgtccaacgaatgggcctaagatcccgtccatcgccactgggatggtgggggccctcctcttgctgctggtggtggccctggggatcggcctcttcatgtga

SEQ ID NO: 17 - DNA, 20 bp, synthetic construct
  misc_feature 1..20: note = SMCO2 gRNA1
  source 1..20: mol_type = other DNA
catccgatctgtctaagatg

SEQ ID NO: 18 - DNA, 20 bp, synthetic construct
  misc_feature 1..20: note = SMCO2 gRNA2
  source 1..20: mol_type = other DNA
tgcagagatgtagacgcttg

SEQ ID NO: 19 - DNA, 20 bp, synthetic construct
  misc_feature 1..20: note = TSR2 gRNA1
  source 1..20: mol_type = other DNA
cttcgggggtgtgcacagcc

SEQ ID NO: 20 - DNA, 20 bp, synthetic construct
  misc_feature 1..20: note = TSR2 gRNA2
  source 1..20: mol_type = other DNA
cacaactgtatcaaactcgt

SEQ ID NO: 21 - DNA, 20 bp, synthetic construct
  misc_feature 1..20: note = PKM gRNA1
  source 1..20: mol_type = other DNA
cctggagcacatgtgccgcc

SEQ ID NO: 22 - DNA, 20 bp, synthetic construct
  misc_feature 1..20: note = PKM gRNA2
  source 1..20: mol_type = other DNA
gacgagctgtctggggattc

SEQ ID NO: 23 - DNA, 20 bp, synthetic construct
  misc_feature 1..20: note = CUL5 gRNA1
  source 1..20: mol_type = other DNA
taacctttgttctaatcctg

SEQ ID NO: 24 - DNA, 20 bp, synthetic construct
  misc_feature 1..20: note = CUL5 gRNA2
  source 1..20: mol_type = other DNA
agcttgtttacataatccgc

SEQ ID NO: 25 - DNA, 20 bp, synthetic construct
  misc_feature 1..20: note = KLRC1 gRNA1
  source 1..20: mol_type = other DNA
ggtctgagtagattactcct

SEQ ID NO: 26 - DNA, 20 bp, synthetic construct
  misc_feature 1..20: note = KLRC1 gRNA2
  source 1..20: mol_type = other DNA
ctgaatacaagaactcagaa

SEQ ID NO: 27 - DNA, 20 bp, synthetic construct
  misc_feature 1..20: note = ING3 gRNA1
  source 1..20: mol_type = other DNA
catccgatctgtctaagatg

SEQ ID NO: 28 - DNA, 20 bp, synthetic construct
  misc_feature 1..20: note = ING3 gRNA2
  source 1..20: mol_type = other DNA
tgattacaaatgcagtatcg

SEQ ID NO: 29 - DNA, 53 bp, synthetic construct
  misc_feature 1..53: note = CUL5 shRNA
  source 1..53: mol_type = other DNA
gctagaatgtttcaggacatactcgagtatgtcctgaaacattctagcttttt

SEQ ID NO: 30 - protein, 42 aa, synthetic construct
KRGRKKLLYIFKQPFMRPVQTTQEEDGCSCRFPEEEEGGCEL

SEQ ID NO: 31 - protein, 61 aa, synthetic construct
RKRWQNEKLGLDAGDEYEDENLYEGLNLDDCSMYEDISRGLQGTYQDVGSLNIGDVQLEKP

SEQ ID NO: 32 - protein, 62 aa, synthetic construct
KKVAKKPTNKAPHPKQEPQEINFPDDLPGSNTAAPVQETLHGCQPVTQEDGKESRISVQERQ

SEQ ID NO: 33 - DNA, 126 bp, synthetic construct
  source 1..126: mol_type = other DNA
aaacggggcagaaagaaactcctgtatatattcaaacaaccatttatgagaccagtacaaactactcaagaggaagatggctgtagctgccgatttccagaagaagaagaaggaggatgtgaactg

SEQ ID NO: 34 - DNA, 183 bp, synthetic construct
  source 1..183: mol_type = other DNA
aggaaacgatggcagaacgagaagctcgggttggatgccggggatgaatatgaagatgaaaacctttatgaaggcctgaacctggacgactgctccatgtatgaggacatctcccggggcctccagggcacctaccaggatgtgggcagcctcaacataggagatgtccagctggagaagccg

SEQ ID NO: 35 - DNA, 186 bp, synthetic construct
  source 1..186: mol_type = other DNA
aaaaaggtggccaagaagccaaccaataaggccccccaccccaagcaggaaccccaggagatcaattttcccgacgatcttcctggctccaacactgctgctccagtgcaggagactttacatggatgccaaccggtcacccaggaggatggcaaagagagtcgcatctcagtgcaggagagacag